European Patent Specification EP 3 856 147 B1, published September 17, 2025. Title: METHODS AND PROBIOTIC COMPOSITIONS FOR THE TREATMENT OF BONE DISORDERS. Applicant: RESEARCH DEVELOPMENT FOUNDATION. The sequence listing filed with the application follows.

SEQUENCE LISTING (22 sequences)

SEQ ID NO: 1 - DNA, 20 bp, Artificial sequence
  Synthetic primer
  misc_feature (8)..(8): n is a, c, g, or t
ggactacnvgggtwtctaat

SEQ ID NO: 2 - DNA, 19 bp, Artificial sequence
  Synthetic primer
gtgycagcmgccgcggtaa

SEQ ID NO: 3 - DNA, 20 bp, Artificial sequence
  Synthetic primer
gcattcagaggcaaatcagc

SEQ ID NO: 4 - DNA, 21 bp, Artificial sequence
  Synthetic primer
gccacacctccagtcattaag

SEQ ID NO: 5 - DNA, 21 bp, Artificial sequence
  Synthetic primer
tgctcttctgtatcgcccagt

SEQ ID NO: 6 - DNA, 21 bp, Artificial sequence
  Synthetic primer
gccgtgttaaggaatctgctg

SEQ ID NO: 7 - DNA, 19 bp, Artificial sequence
  Synthetic primer
ccctgccattgttaagacc

SEQ ID NO: 8 - DNA, 19 bp, Artificial sequence
  Synthetic primer
tgctgctgttcctgttttc

SEQ ID NO: 9 - DNA, 23 bp, Artificial sequence
  Synthetic primer
cagtgtggtgcacgtctccaatc

SEQ ID NO: 10 - DNA, 21 bp, Artificial sequence
  Synthetic primer
tgaaccaaagttgaccaccag

SEQ ID NO: 11 - DNA, 21 bp, Artificial sequence
  Synthetic primer
gaagctgcggtacaattccag

SEQ ID NO: 12 - DNA, 21 bp, Artificial sequence
  Synthetic primer
ccccttgtacccttcaccaat

SEQ ID NO: 13 - DNA, 19 bp, Artificial sequence
  Synthetic primer
ttgtctcactgaccggcct

SEQ ID NO: 14 - DNA, 22 bp, Artificial sequence
  Synthetic primer
tatgttcggcttcccattctcc

SEQ ID NO: 15 - DNA, 23 bp, Artificial sequence
  Synthetic primer
gggttcctataaatacggactgc

SEQ ID NO: 16 - DNA, 20 bp, Artificial sequence
  Synthetic primer
ccattttgtctacgggacga

SEQ ID NO: 17 - DNA, 20 bp, Artificial sequence
  Synthetic primer
agagccccatctgtcctctc

SEQ ID NO: 18 - DNA, 22 bp, Artificial sequence
  Synthetic primer
actggtagtctgcaaaaccaaa

SEQ ID NO: 19 - DNA, 18 bp, Artificial sequence
  Synthetic primer
cagcacggtgaagccatt

SEQ ID NO: 20 - DNA, 17 bp, Artificial sequence
  Synthetic primer
gcgtgcatccgcttgtg

SEQ ID NO: 21 - DNA, 22 bp, Artificial sequence
  Synthetic primer
cctgtcagtcttggcctatgag

SEQ ID NO: 22 - DNA, 20 bp, Artificial sequence
  Synthetic primer
gcccaatgagatgagcgata